European Patent Application EP 4 686 476 A1, published February 4, 2026. Title: SUBSTANCE OR COMPOSITION COMPRISING A COMPOUND FOR NEUROLOGICAL DISORDERS AND TESTSYSTEM ALLOWING TO TEST SUITABLE SUBSTANCES OR COMPOSITIONS. Applicant: Klostermeier. Application EP. The sequence listing filed with the application follows.

SEQUENCE LISTING (22 sequences)

SEQ ID NO: 1 - DNA, 20 bp, synthetic construct
  source 1..20: mol_type = other DNA
atcgccatcatctggttccc

SEQ ID NO: 2 - DNA, 20 bp, synthetic construct
  source 1..20: mol_type = other DNA
tggtgaacagcggctcatag

SEQ ID NO: 3 - DNA, 23 bp, synthetic construct
  source 1..23: mol_type = other DNA
catggtgaaacgcataagaatca

SEQ ID NO: 4 - DNA, 20 bp, synthetic construct
  source 1..20: mol_type = other DNA
caacccaagccagaccaagt

SEQ ID NO: 5 - DNA, 19 bp, synthetic construct
  source 1..19: mol_type = other DNA
cacagcatctccaggagcc

SEQ ID NO: 6 - DNA, 19 bp, synthetic construct
  source 1..19: mol_type = other DNA
gtgtccctggcttctgtcc

SEQ ID NO: 7 - DNA, 20 bp, synthetic construct
  source 1..20: mol_type = other DNA
aggtcggagtcaacggattt

SEQ ID NO: 8 - DNA, 20 bp, synthetic construct
  source 1..20: mol_type = other DNA
tggaatttgccatgggtgga

SEQ ID NO: 9 - DNA, 23 bp, synthetic construct
  source 1..23: mol_type = other DNA
ggccgaatataacatagagccac

SEQ ID NO: 10 - DNA, 21 bp, synthetic construct
  source 1..21: mol_type = other DNA
tgaacaagctcttcaggtggt

SEQ ID NO: 11 - DNA, 20 bp, synthetic construct
  source 1..20: mol_type = other DNA
cttcggcattctgcaacagt

SEQ ID NO: 12 - DNA, 21 bp, synthetic construct
  source 1..21: mol_type = other DNA
gcctagtcttcaactggtgtg

SEQ ID NO: 13 - DNA, 21 bp, synthetic construct
  source 1..21: mol_type = other DNA
cctccttgaggatgaggctga

SEQ ID NO: 14 - DNA, 20 bp, synthetic construct
  source 1..20: mol_type = other DNA
cgacctgaagctgttcctgg

SEQ ID NO: 15 - DNA, 21 bp, synthetic construct
  source 1..21: mol_type = other DNA
cacccattcaaatggagcacg

SEQ ID NO: 16 - DNA, 19 bp, synthetic construct
  source 1..19: mol_type = other DNA
gcagctgtggagggtagtg

SEQ ID NO: 17 - DNA, 15 bp, synthetic construct
  source 1..15: mol_type = other DNA
cccggaggctgagca

SEQ ID NO: 18 - DNA, 20 bp, synthetic construct
  source 1..20: mol_type = other DNA
tcaaacagattggccaggga

SEQ ID NO: 19 - DNA, 20 bp, synthetic construct
  source 1..20: mol_type = other DNA
gagtatgcctgccgtgtgaa

SEQ ID NO: 20 - DNA, 20 bp, synthetic construct
  source 1..20: mol_type = other DNA
cggcatcttcaaacctccat

SEQ ID NO: 21 - DNA, 20 bp, synthetic construct
  source 1..20: mol_type = other DNA
cctggcgtcgtgattagtga

SEQ ID NO: 22 - DNA, 20 bp, synthetic construct
  source 1..20: mol_type = other DNA
cgagcaagacgttcagtcct